European Patent Application EP 4 549 583 A1, published May 7, 2025. Title: 블로커 핵산 처리를 포함하는 표적 RNA 검출 방법. Applicant: 주식회사 제노헬릭스. Application KR. The sequence listing filed with the application follows.

SEQUENCE LISTING (13 sequences)

SEQ ID NO: 1 - DNA, 20 bp, synthetic construct
  source 1..20: mol_type = other DNA
tgagtgggcactccgctgcc

SEQ ID NO: 2 - DNA, 167 bp, synthetic construct
  source 1..167: mol_type = other DNA
aacaataccacgaccaccgactgaaagggtggatcgtgaagggggcttcttgttggacagtcagtggatgctcaaggccagggcagcggagtgcccactcagatctgctccttgtgcttcagttgcttggctctggtgtattggtacaggccgggacaagtgcaata

SEQ ID NO: 3 - DNA, 200 bp, synthetic construct
  source 1..200: mol_type = other DNA
aacaataccacgaccaccgacgtgcttggagtcaatcggatgtaggatggtctccagacaccggaccactcttcacgcctaaagcataaacgtcgagcagtggcagcggagtgcccactcagaaagtcttagtaccggacgtgccgtttcactgcggttgcttggctctggtgtattggtagtacatcatctatactgta

SEQ ID NO: 4 - DNA, 187 bp, synthetic construct
  source 1..187: mol_type = other DNA
aacaataccacgaccaccgacgagggcacaatcctattcccatttgtatgttcagctaacttctacccatccccggcagcggagtgcccactcagttaagtaggtcgtgagatgccatggaggctctcgttcatcccgtgggttgcttggctctggtgtattggtaactatgcaacctactacctct

SEQ ID NO: 5 - DNA, 20 bp, synthetic construct
  source 1..20: mol_type = other DNA
tgaaagggtggatcgtgaag

SEQ ID NO: 6 - DNA, 21 bp, synthetic construct
  source 1..21: mol_type = other DNA
taccaatacaccagagccaag

SEQ ID NO: 7 - DNA, 23 bp, synthetic construct
  source 1..23: mol_type = other DNA
agtcagtggatgctcaaggccag

SEQ ID NO: 8 - DNA, 22 bp, synthetic construct
  source 1..22: mol_type = other DNA
cttggagtcaatcggatgtagg

SEQ ID NO: 9 - DNA, 22 bp, synthetic construct
  source 1..22: mol_type = other DNA
cacgtccggtactaagactttc

SEQ ID NO: 10 - DNA, 26 bp, synthetic construct
  source 1..26: mol_type = other DNA
cgcctaaagcataaacgtcgagcagt

SEQ ID NO: 11 - DNA, 22 bp, synthetic construct
  source 1..22: mol_type = other DNA
ggcacaatcctattcccatttg

SEQ ID NO: 12 - DNA, 22 bp, synthetic construct
  source 1..22: mol_type = other DNA
ggcatctcacgacctacttaac

SEQ ID NO: 13 - DNA, 27 bp, synthetic construct
  source 1..27: mol_type = other DNA
atgttcagctaacttctacccatcccc